European Patent Specification EP 3 700 559 B1, published August 26, 2026. Title: Single strain dysentery vaccine. Applicant: Aquilon CYL S.L. The sequence listing filed with the application follows.

SEQUENCE LISTING (6 sequences)

SEQ ID NO: 1 - DNA, 775 bp, Brachyspira hyodysenteriae
  TlyA (tlyA) gene, partial cds, GenBank: KU215622.1
gtaaatatgagagataaagaaagaaattctctttctataataaaatctttccttggattataatactaatataaatgcgattagatgaatatgtgcatagtgaaggctatacagaaagcagatctaaagcacaggatataatactagccggttgtgtttttgttaatggagtaaaggtaacttctaaggctcataaaataaaagatactgataatatagaagttgttcagaatataaaatatgtatcaagagctggagaaaaattagaaaaggcgtttgtagaatttggaatatctgtagaaaataaaatatgtttagatataggagcttctacaggaggatttacagattgtctgcttaagcatggtgctaaaaaagtttatgctcttgatgtaggacataatcagctagtttataaacttcgtaatgataatagggtagtgtcaatagaagatttcaatgccaaagatataaataaagaaatgttcaatgatgaaatcccatctgtaatagtaagtgacgtatcatttatatcaataacaaaaatagcaccaatcatatttaaagaattaaataatttagagttttgggtaactttaataaaaccacaatttgaagctgaaagaggtgatgtttcaaaaggcggtataatacgagatgatatacttagagaaaaaatattaaataatgctatttcaaagataatagactgcggatttaaagaagttaatagaaccatctctcctataaaaggtgctaaaggtaatatagaata

SEQ ID NO: 2 - DNA, 20 bp, Artificial Sequence
  Bh tlyA_F primer
gcagatctaaagcacaggat

SEQ ID NO: 3 - DNA, 20 bp, Artificial Sequence
  Bh tlyA_R primer
gccttttgaaacatcacctc

SEQ ID NO: 4 - DNA, 1346 bp, Brachyspira pilosicoli
  gene for 16S ribosomal RNA, partial sequence
atgcagtcgagcgggcttattcgggcaactggataagttagcggcgaactggtgagtaacacgtaggtaatctgccgtgaagtgggggataacccatggaaacatggactaataccgcatatactcttgctacataagtagagtagaggaaagttttttcgcttcacgatgagcctgcggcctattagcctgttggtagggtaatggcctaccaaagctacgataggtagccgacctgagagggtgaccggccacattgggactgagatacggcccagactcctacgggaggcagcagctgagaatcttccacaatggacgaaagtctgatggagcgacatcgcgtgagggatgaaggccttcgggttgtaaacctcggaaattatcgaagaatgagtgacagtagataatgtaagcctcggctaactacgtgccagcagccgcggtaatacgtaggaggcaaacgttgctcggatttactgggcgtaaagggtgagtaggcggatttataagtctaaggtgaaagaccgaagctcaacttcgggaacgcctcggatactgtaagtcttggatattgtaggggatgatggaattctcggtgtagcggtggaatgcgcagatatcgagaggaacacctatagcgaaggcagtcatctgggcatttatcgacgctgaatcacgaaagctaggggagcaaacaggcttagataccctggtagtcctagccgtaaacgttgtacactaggtgcttctatttaaataggagtgccgtagctaacgtcttaagtgtaccgcctgaggagtatgcccgcaagggtgaaactcaaagaaattgacgggtccccgcacaagtggtggagcatgtggtttaattcgatgatacgcgaaaaaccttacctgggtttgaattgttagatgaatgatttagagataagtcagaccgcaaggacgtttaacataggtgctgcatggctgtcgtcagctcgtgtcgtgagatgttgggttaagtcccgcaacgagcgcaaccctcaccctctgttgctaacgagtaatgtcgagcactcttaggggactgcctacgttcaagtaggaggaaggtggggatgatgtcaagtcctcatggcccttatgtccagggctacacacgtgctacaatggcaagtacaaagagaagcaagaccgcgaggtggagcaaaactcaaaaaagttgcctcagttcggattggagtctgaaactcgactccatgaagttggaatcactagtaatcgtagatcagaacgctacggtgaatacgttcccggggattgtacacaccgcccgtcacgccatcggagttggttttacc

SEQ ID NO: 5 - DNA, 26 bp, Artificial Sequence
  Bp16S_ F: 5 primer
cataagtagagtagaggaaagttttt

SEQ ID NO: 6 - DNA, 24 bp, Artificial Sequence
  Bp16S_R: 5 primer
ctcgacattactcggtagcaacag